European Patent Specification EP 3 825 400 B1, published December 25, 2024. Title: MULTIMERIC CODING NUCLEIC ACID AND USES THEREOF. Applicant: RANA THERAPEUTICS, INC. The sequence listing filed with the application follows.

SEQUENCE LISTING (26 sequences)

SEQ ID NO: 1 - RNA, 827 nt, Artificial Sequence
  Chemically synthesized nucleotide
ggacagaucgccuggagacgccauccacgcuguuuugaccuccauagaagacaccgggaccgauccagccuccgcggccgggaacggugcauuggaacgcggauuccccgugccaagagugacucaccguccuugacacgaugggggugcacgaauguccugccuggcuguggcuucuccugucccugcugucgcucccucugggccucccaguccugggcgccccaccacgccucaucugugacagccgaguccuggagagguaccucuuggaggccaaggaggccgagaauaucacgacgggcugugcugaacacugcagcuugaaugagaauaucacugucccagacaccaaaguuaauuucuaugccuggaagaggauggaggucgggcagcaggccguagaagucuggcagggccuggcccugcugucggaagcuguccugcggggccaggcccuguuggucaacucuucccagccgugggagccccugcagcugcauguggauaaagccgucaguggccuucgcagccucaccacucugcuucgggcucugggagcccagaaggaagccaucuccccuccagaugcggccucagcugcuccacuccgaacaaucacugcugacacuuuccgcaaacucuuccgagucuacuccaauuuccuccggggaaagcugaagcuguacacaggggaggccugcaggacaggggacagaugacggguggcaucccugugaccccuccccagugccucuccuggcccuggaaguugccacuccagugcccaccagccuuguccuaauaaaauuaaguugcaucaagcu

SEQ ID NO: 2 - RNA, 1027 nt, Artificial Sequence
  Chemically synthesized nucleotide
ggacagaucgccuggagacgccauccacgcuguuuugaccuccauagaagacaccgggaccgauccagccuccgcggccgggaacggugcauuggaacgcggauuccccgugccaagagugacucaccguccuugacacgaugggggugcacgaauguccugccuggcuguggcuucuccugucccugcugucgcucccucugggccucccaguccugggcgccccaccacgccucaucugugacagccgaguccuggagagguaccucuuggaggccaaggaggccgagaauaucacgacgggcugugcugaacacugcagcuugaaugagaauaucacugucccagacaccaaaguuaauuucuaugccuggaagaggauggaggucgggcagcaggccguagaagucuggcagggccuggcccugcugucggaagcuguccugcggggccaggcccuguuggucaacucuucccagccgugggagccccugcagcugcauguggauaaagccgucaguggccuucgcagccucaccacucugcuucgggcucugggagcccagaaggaagccaucuccccuccagaugcggccucagcugcuccacuccgaacaaucacugcugacacuuuccgcaaacucuuccgagucuacuccaauuuccuccggggaaagcugaagcuguacacaggggaggccugcaggacaggggacagaugacggguggcaucccugugaccccuccccagugccucuccuggcccuggaaguugccacuccagugcccaccagccuuguccuaauaaaauuaaguugcaucaagcuaaaaaaaaaaaaaaaaaaaaaaaaaaaaaaaaaaaaaaaaaaaaaaaaaaaaaaaaaaaaaaaaaaaaaaaaaaaaaaaaaaaaaaaaaaaaaaaaaaaaaaaaaaaaaaaaaaaaaaaaaaaaaaaaaaaaaaaaaaaaaaaaaaaaaaaaaaaaaaaaaaaaaaaaaaaaaaaaaaaaaaaaaaaaaaaaaaaaaaaa

SEQ ID NO: 3 - RNA, 891 nt, Artificial Sequence
  Chemically synthesized nucleotide
ggacagaucgccuggagacgccauccacgcuguuuugaccuccauagaagacaccgggaccgauccagccuccgcggccgggaacggugcauuggaacgcggauuccccgugccaagagugacucaccguccuugacacgaugggggugcacgaauguccugccuggcuguggcuucuccugucccugcugucgcucccucugggccucccaguccugggcgccccaccacgccucaucugugacagccgaguccuggagagguaccucuuggaggccaaggaggccgagaauaucacgacgggcugugcugaacacugcagcuugaaugagaauaucacugucccagacaccaaaguuaauuucuaugccuggaagaggauggaggucgggcagcaggccguagaagucuggcagggccuggcccugcugucggaagcuguccugcggggccaggcccuguuggucaacucuucccagccgugggagccccugcagcugcauguggauaaagccgucaguggccuucgcagccucaccacucugcuucgggcucugggagcccagaaggaagccaucuccccuccagaugcggccucagcugcuccacuccgaacaaucacugcugacacuuuccgcaaacucuuccgagucuacuccaauuuccuccggggaaagcugaagcuguacacaggggaggccugcaggacaggggacagaugacggguggcaucccugugaccccuccccagugccucuccuggcccuggaaguugccacuccagugcccaccaaaaaaaaaaaaaaaaaaaaaaaaaaaaaaaaaaaaaaaaaaaaaaaaaaaaaaaaaaaaaaaaagccuuguccuaauaaaauuaaguugcaucaagcu

SEQ ID NO: 4 - RNA, 883 nt, Artificial Sequence
  Chemically synthesized nucleotide
ggacagaucgccuggagacgccauccacgcuguuuugaccuccauagaagacaccgggaccgauccagccuccgcggccgggaacggugcauuggaacgcggauuccccgugccaagagugacucaccguccuugacacgaugggggugcacgaauguccugccuggcuguggcuucuccugucccugcugucgcucccucugggccucccaguccugggcgccccaccacgccucaucugugacagccgaguccuggagagguaccucuuggaggccaaggaggccgagaauaucacgacgggcugugcugaacacugcagcuugaaugagaauaucacugucccagacaccaaaguuaauuucuaugccuggaagaggauggaggucgggcagcaggccguagaagucuggcagggccuggcccugcugucggaagcuguccugcggggccaggcccuguuggucaacucuucccagccgugggagccccugcagcugcauguggauaaagccgucaguggccuucgcagccucaccacucugcuucgggcucugggagcccagaaggaagccaucuccccuccagaugcggccucagcugcuccacuccgaacaaucacugcugacacuuuccgcaaacucuuccgagucuacuccaauuuccuccggggaaagcugaagcuguacacaggggaggccugcaggacaggggacagaugacggguggcaaaaaaaaaaaaaaaucccugugaccccuccccaaaaaaaaaaaaaaaagugccucuccuggcccuggaaaaaaaaaaaaaaaguugccacuccagugcccaccaaaaaaaaaaaaaaagccuuguccuaauaaaauuaaguugcaucaagcu

SEQ ID NO: 5 - RNA, 20 nt, Artificial Sequence
  Chemically synthesized nucleotide
  MISC_FEATURE (10)..(11): 3'-3' bridge between nucleotides at positions 10 and 11 comprises PO4
cgacucucggggcucucagc

SEQ ID NO: 6 - RNA, 20 nt, Artificial Sequence
  Chemically synthesized nucleotide
  MISC_FEATURE (10)..(11): 3'-3' bridge between nucleotides at positions 10 and 11 comprises PO4
aaaaaaaaaaaaaaaaaaaa

SEQ ID NO: 7 - RNA, 6 nt, Artificial Sequence
  Chemically synthesized nucleotide
  MISC_FEATURE (3)..(4): 3'-3' bridge between nucleotides at positions 3 and 4 comprises PO4
aaaaaa

SEQ ID NO: 8 - RNA, 2 nt, Artificial Sequence
  Chemically synthesized nucleotide
  MISC_FEATURE (1)..(2): 3'-3' bridge between nucleotides at positions 1 and 2 comprises PO4
aa

SEQ ID NO: 9 - DNA, 37 bp, Artificial Sequence
  Chemically synthesized nucleotide
ccgagagtcgagcttgatgcaacttaattttattagg

SEQ ID NO: 10 - DNA, 30 bp, Artificial Sequence
  Chemically synthesized nucleotide
ccgagagtgatgcaacttaattttattagg

SEQ ID NO: 11 - DNA, 37 bp, Artificial Sequence
  Chemically synthesized nucleotide
ttttttttttagcttgatgcaacttaattttattagg

SEQ ID NO: 12 - DNA, 30 bp, Artificial Sequence
  Chemically synthesized nucleotide
ccgagagtcgtttttttttttttttttttt

SEQ ID NO: 13 - DNA, 74 bp, Artificial Sequence
  Chemically synthesized nucleotide
  misc_feature (37)..(38): 5'-5' bridge between nucleotides at positions 37 and 38 comprises PO4
ggattattttaattcaacgtagttcgagctgagagccccgagagtcgagcttgatgcaacttaattttattagg

SEQ ID NO: 14 - DNA, 60 bp, Artificial Sequence
  Chemically synthesized nucleotide
  misc_feature (30)..(31): 5'-5' bridge between nucleotides at positions 30 and 31 comprises PO4
ggattattttaattcaacgtagtgagagccccgagagtgatgcaacttaattttattagg

SEQ ID NO: 15 - DNA, 74 bp, Artificial Sequence
  Chemically synthesized nucleotide
  misc_feature (37)..(38): 5'-5' bridge between nucleotides at positions 37 and 38 comprises PO4
ggattattttaattcaacgtagttcgattttttttttttttttttttagcttgatgcaacttaattttattagg

SEQ ID NO: 16 - DNA, 60 bp, Artificial Sequence
  Chemically synthesized nucleotide
  misc_feature (30)..(31): 5'-5' bridge between nucleotides at positions 30 and 31 comprises PO4
ttttttttttttttttttttgctgagagccccgagagtcgtttttttttttttttttttt

SEQ ID NO: 17 - RNA, 1674 nt, Artificial Sequence
  Chemically synthesized nucleotide
  misc_feature (837)..(838): 3'-3' bridge between nucleotides at positions 837 and 838 comprises PO4
ggacagaucgccuggagacgccauccacgcuguuuugaccuccauagaagacaccgggaccgauccagccuccgcggccgggaacggugcauuggaacgcggauuccccgugccaagagugacucaccguccuugacacgaugggggugcacgaauguccugccuggcuguggcuucuccugucccugcugucgcucccucugggccucccaguccugggcgccccaccacgccucaucugugacagccgaguccuggagagguaccucuuggaggccaaggaggccgagaauaucacgacgggcugugcugaacacugcagcuugaaugagaauaucacugucccagacaccaaaguuaauuucuaugccuggaagaggauggaggucgggcagcaggccguagaagucuggcagggccuggcccugcugucggaagcuguccugcggggccaggcccuguuggucaacucuucccagccgugggagccccugcagcugcauguggauaaagccgucaguggccuucgcagccucaccacucugcuucgggcucugggagcccagaaggaagccaucuccccuccagaugcggccucagcugcuccacuccgaacaaucacugcugacacuuuccgcaaacucuuccgagucuacuccaauuuccuccggggaaagcugaagcuguacacaggggaggccugcaggacaggggacagaugacggguggcaucccugugaccccuccccagugccucuccuggcccuggaaguugccacuccagugcccaccagccuuguccuaauaaaauuaaguugcaucaagcucgacucucggggcucucagcucgaacuacguugaauuaaaauaauccuguuccgaccacccgugaccucaccguugaaggucccgguccucuccgugaccccuccccagugucccuacggugggcaguagacaggggacaggacguccggaggggacacaugucgaagucgaaaggggccuccuuuaaccucaucugagccuucucaaacgccuuucacagucgucacuaacaagccucaccucgucgacuccggcguagaccuccccucuaccgaaggaagacccgagggucucgggcuucgucucaccacuccgacgcuuccggugacugccgaaauagguguacgucgacguccccgagggugccgacccuucucaacugguugucccggaccggggcguccugucgaaggcugucgucccgguccgggacggucugaagaugccggacgacgggcuggagguaggagaagguccguaucuuuaauugaaaccacagacccugucacuauaagaguaaguucgacgucacaagucgugucgggcagcacuauaagagccggaggaaccggagguucuccauggagagguccugagccgacagugucuacuccgcaccaccccgcggguccugacccuccgggucucccucgcugucgucccuguccucuucggugucgguccguccuguaagcacguggggguagcacaguuccugccacucagugagaaccgugccccuuaggcgcaagguuacguggcaagggccggcgccuccgaccuagccagggccacagaagauaccuccaguuuugucgcaccuaccgcagagguccgcuagacagg

SEQ ID NO: 18 - RNA, 1674 nt, Artificial Sequence
  Chemically synthesized nucleotide
  misc_feature (837)..(838): 3'-3' bridge between nucleotides at positions 837 and 838 comprises PO4
ggacagaucgccuggagacgccauccacgcuguuuugaccuccauagaagacaccgggaccgauccagccuccgcggccgggaacggugcauuggaacgcggauuccccgugccaagagugacucaccguccuugacacgaugggggugcacgaauguccugccuggcuguggcuucuccugucccugcugucgcucccucugggccucccaguccugggcgccccaccacgccucaucugugacagccgaguccuggagagguaccucuuggaggccaaggaggccgagaauaucacgacgggcugugcugaacacugcagcuugaaugagaauaucacugucccagacaccaaaguuaauuucuaugccuggaagaggauggaggucgggcagcaggccguagaagucuggcagggccuggcccugcugucggaagcuguccugcggggccaggcccuguuggucaacucuucccagccgugggagccccugcagcugcauguggauaaagccgucaguggccuucgcagccucaccacucugcuucgggcucugggagcccagaaggaagccaucuccccuccagaugcggccucagcugcuccacuccgaacaaucacugcugacacuuuccgcaaacucuuccgagucuacuccaauuuccuccggggaaagcugaagcuguacacaggggaggccugcaggacaggggacagaugacggguggcaucccugugaccccuccccagugccucuccuggcccuggaaguugccacuccagugcccaccagccuuguccuaauaaaauuaaguugcaucaagcuaaaaaaaaaaaaaaaaaaaaucgaacuacguugaauuaaaauaauccuguuccgaccacccgugaccucaccguugaaggucccgguccucuccgugaccccuccccagugucccuacggugggcaguagacaggggacaggacguccggaggggacacaugucgaagucgaaaggggccuccuuuaaccucaucugagccuucucaaacgccuuucacagucgucacuaacaagccucaccucgucgacuccggcguagaccuccccucuaccgaaggaagacccgagggucucgggcuucgucucaccacuccgacgcuuccggugacugccgaaauagguguacgucgacguccccgagggugccgacccuucucaacugguugucccggaccggggcguccugucgaaggcugucgucccgguccgggacggucugaagaugccggacgacgggcuggagguaggagaagguccguaucuuuaauugaaaccacagacccugucacuauaagaguaaguucgacgucacaagucgugucgggcagcacuauaagagccggaggaaccggagguucuccauggagagguccugagccgacagugucuacuccgcaccaccccgcggguccugacccuccgggucucccucgcugucgucccuguccucuucggugucgguccguccuguaagcacguggggguagcacaguuccugccacucagugagaaccgugccccuuaggcgcaagguuacguggcaagggccggcgccuccgaccuagccagggccacagaagauaccuccaguuuugucgcaccuaccgcagagguccgcuagacagg

SEQ ID NO: 19 - RNA, 2074 nt, Artificial Sequence
  Chemically synthesized nucleotide
  misc_feature (1037)..(1038): 3'-3' bridge between nucleotides at positions 1037 and 1038 comprises PO4
ggacagaucgccuggagacgccauccacgcuguuuugaccuccauagaagacaccgggaccgauccagccuccgcggccgggaacggugcauuggaacgcggauuccccgugccaagagugacucaccguccuugacacgaugggggugcacgaauguccugccuggcuguggcuucuccugucccugcugucgcucccucugggccucccaguccugggcgccccaccacgccucaucugugacagccgaguccuggagagguaccucuuggaggccaaggaggccgagaauaucacgacgggcugugcugaacacugcagcuugaaugagaauaucacugucccagacaccaaaguuaauuucuaugccuggaagaggauggaggucgggcagcaggccguagaagucuggcagggccuggcccugcugucggaagcuguccugcggggccaggcccuguuggucaacucuucccagccgugggagccccugcagcugcauguggauaaagccgucaguggccuucgcagccucaccacucugcuucgggcucugggagcccagaaggaagccaucuccccuccagaugcggccucagcugcuccacuccgaacaaucacugcugacacuuuccgcaaacucuuccgagucuacuccaauuuccuccggggaaagcugaagcuguacacaggggaggccugcaggacaggggacagaugacggguggcaucccugugaccccuccccagugccucuccuggcccuggaaguugccacuccagugcccaccagccuuguccuaauaaaauuaaguugcaucaagcuaaaaaaaaaaaaaaaaaaaaaaaaaaaaaaaaaaaaaaaaaaaaaaaaaaaaaaaaaaaaaaaaaaaaaaaaaaaaaaaaaaaaaaaaaaaaaaaaaaaaaaaaaaaaaaaaaaaaaaaaaaaaaaaaaaaaaaaaaaaaaaaaaaaaaaaaaaaaaaaaaaaaaaaaaaaaaaaaaaaaaaaaaaaaaaaaaaaaaaaacgacucucggggcucucagcaaaaaaaaaaaaaaaaaaaaaaaaaaaaaaaaaaaaaaaaaaaaaaaaaaaaaaaaaaaaaaaaaaaaaaaaaaaaaaaaaaaaaaaaaaaaaaaaaaaaaaaaaaaaaaaaaaaaaaaaaaaaaaaaaaaaaaaaaaaaaaaaaaaaaaaaaaaaaaaaaaaaaaaaaaaaaaaaaaaaaaaaaaaaaaaaaaaaaaaaucgaacuacguugaauuaaaauaauccuguuccgaccacccgugaccucaccguugaaggucccgguccucuccgugaccccuccccagugucccuacggugggcaguagacaggggacaggacguccggaggggacacaugucgaagucgaaaggggccuccuuuaaccucaucugagccuucucaaacgccuuucacagucgucacuaacaagccucaccucgucgacuccggcguagaccuccccucuaccgaaggaagacccgagggucucgggcuucgucucaccacuccgacgcuuccggugacugccgaaauagguguacgucgacguccccgagggugccgacccuucucaacugguugucccggaccggggcguccugucgaaggcugucgucccgguccgggacggucugaagaugccggacgacgggcuggagguaggagaagguccguaucuuuaauugaaaccacagacccugucacuauaagaguaaguucgacgucacaagucgugucgggcagcacuauaagagccggaggaaccggagguucuccauggagagguccugagccgacagugucuacuccgcaccaccccgcggguccugacccuccgggucucccucgcugucgucccuguccucuucggugucgguccguccuguaagcacguggggguagcacaguuccugccacucagugagaaccgugccccuuaggcgcaagguuacguggcaagggccggcgccuccgaccuagccagggccacagaagauaccuccaguuuugucgcaccuaccgcagagguccgcuagacagg

SEQ ID NO: 20 - RNA, 2060 nt, Artificial Sequence
  Chemically synthesized nucleotide
  misc_feature (1030)..(1031): 3'-3' bridge between nucleotides at positions 1030 and 1031 comprises PO4
ggacagaucgccuggagacgccauccacgcuguuuugaccuccauagaagacaccgggaccgauccagccuccgcggccgggaacggugcauuggaacgcggauuccccgugccaagagugacucaccguccuugacacgaugggggugcacgaauguccugccuggcuguggcuucuccugucccugcugucgcucccucugggccucccaguccugggcgccccaccacgccucaucugugacagccgaguccuggagagguaccucuuggaggccaaggaggccgagaauaucacgacgggcugugcugaacacugcagcuugaaugagaauaucacugucccagacaccaaaguuaauuucuaugccuggaagaggauggaggucgggcagcaggccguagaagucuggcagggccuggcccugcugucggaagcuguccugcggggccaggcccuguuggucaacucuucccagccgugggagccccugcagcugcauguggauaaagccgucaguggccuucgcagccucaccacucugcuucgggcucugggagcccagaaggaagccaucuccccuccagaugcggccucagcugcuccacuccgaacaaucacugcugacacuuuccgcaaacucuuccgagucuacuccaauuuccuccggggaaagcugaagcuguacacaggggaggccugcaggacaggggacagaugacggguggcaucccugugaccccuccccagugccucuccuggcccuggaaguugccacuccagugcccaccagccuuguccuaauaaaauuaaguugcaucaagcuaaaaaaaaaaaaaaaaaaaaaaaaaaaaaaaaaaaaaaaaaaaaaaaaaaaaaaaaaaaaaaaaaaaaaaaaaaaaaaaaaaaaaaaaaaaaaaaaaaaaaaaaaaaaaaaaaaaaaaaaaaaaaaaaaaaaaaaaaaaaaaaaaaaaaaaaaaaaaaaaaaaaaaaaaaaaaaaaaaaaaaaaaaaaaaaaaaaaaaaaaaaaaaaaaaaaaaaaaaaaaaaaaaaaaaaaaaaaaaaaaaaaaaaaaaaaaaaaaaaaaaaaaaaaaaaaaaaaaaaaaaaaaaaaaaaaaaaaaaaaaaaaaaaaaaaaaaaaaaaaaaaaaaaaaaaaaaaaaaaaaaaaaaaaaaaaaaaaaaaaaaaaaaaaaaaaaaaaaaaaaaaaaaaaaaaaaaaaaaaaaaaaaaucgaacuacguugaauuaaaauaauccuguuccgaccacccgugaccucaccguugaaggucccgguccucuccgugaccccuccccagugucccuacggugggcaguagacaggggacaggacguccggaggggacacaugucgaagucgaaaggggccuccuuuaaccucaucugagccuucucaaacgccuuucacagucgucacuaacaagccucaccucgucgacuccggcguagaccuccccucuaccgaaggaagacccgagggucucgggcuucgucucaccacuccgacgcuuccggugacugccgaaauagguguacgucgacguccccgagggugccgacccuucucaacugguugucccggaccggggcguccugucgaaggcugucgucccgguccgggacggucugaagaugccggacgacgggcuggagguaggagaagguccguaucuuuaauugaaaccacagacccugucacuauaagaguaaguucgacgucacaagucgugucgggcagcacuauaagagccggaggaaccggagguucuccauggagagguccugagccgacagugucuacuccgcaccaccccgcggguccugacccuccgggucucccucgcugucgucccuguccucuucggugucgguccguccuguaagcacguggggguagcacaguuccugccacucagugagaaccgugccccuuaggcgcaagguuacguggcaagggccggcgccuccgaccuagccagggccacagaagauaccuccaguuuugucgcaccuaccgcagagguccgcuagacagg

SEQ ID NO: 21 - RNA, 2056 nt, Artificial Sequence
  Chemically synthesized nucleotide
  misc_feature (1028)..(1029): 3'-3' bridge between nucleotides at positions 1028 and 1029 comprises PO4
ggacagaucgccuggagacgccauccacgcuguuuugaccuccauagaagacaccgggaccgauccagccuccgcggccgggaacggugcauuggaacgcggauuccccgugccaagagugacucaccguccuugacacgaugggggugcacgaauguccugccuggcuguggcuucuccugucccugcugucgcucccucugggccucccaguccugggcgccccaccacgccucaucugugacagccgaguccuggagagguaccucuuggaggccaaggaggccgagaauaucacgacgggcugugcugaacacugcagcuugaaugagaauaucacugucccagacaccaaaguuaauuucuaugccuggaagaggauggaggucgggcagcaggccguagaagucuggcagggccuggcccugcugucggaagcuguccugcggggccaggcccuguuggucaacucuucccagccgugggagccccugcagcugcauguggauaaagccgucaguggccuucgcagccucaccacucugcuucgggcucugggagcccagaaggaagccaucuccccuccagaugcggccucagcugcuccacuccgaacaaucacugcugacacuuuccgcaaacucuuccgagucuacuccaauuuccuccggggaaagcugaagcuguacacaggggaggccugcaggacaggggacagaugacggguggcaucccugugaccccuccccagugccucuccuggcccuggaaguugccacuccagugcccaccagccuuguccuaauaaaauuaaguugcaucaagcuaaaaaaaaaaaaaaaaaaaaaaaaaaaaaaaaaaaaaaaaaaaaaaaaaaaaaaaaaaaaaaaaaaaaaaaaaaaaaaaaaaaaaaaaaaaaaaaaaaaaaaaaaaaaaaaaaaaaaaaaaaaaaaaaaaaaaaaaaaaaaaaaaaaaaaaaaaaaaaaaaaaaaaaaaaaaaaaaaaaaaaaaaaaaaaaaaaaaaaaaaaaaaaaaaaaaaaaaaaaaaaaaaaaaaaaaaaaaaaaaaaaaaaaaaaaaaaaaaaaaaaaaaaaaaaaaaaaaaaaaaaaaaaaaaaaaaaaaaaaaaaaaaaaaaaaaaaaaaaaaaaaaaaaaaaaaaaaaaaaaaaaaaaaaaaaaaaaaaaaaaaaaaaaaaaaaaaaaaaaaaaaaaaaaaaaaaaaaaaaaaaucgaacuacguugaauuaaaauaauccuguuccgaccacccgugaccucaccguugaaggucccgguccucuccgugaccccuccccagugucccuacggugggcaguagacaggggacaggacguccggaggggacacaugucgaagucgaaaggggccuccuuuaaccucaucugagccuucucaaacgccuuucacagucgucacuaacaagccucaccucgucgacuccggcguagaccuccccucuaccgaaggaagacccgagggucucgggcuucgucucaccacuccgacgcuuccggugacugccgaaauagguguacgucgacguccccgagggugccgacccuucucaacugguugucccggaccggggcguccugucgaaggcugucgucccgguccgggacggucugaagaugccggacgacgggcuggagguaggagaagguccguaucuuuaauugaaaccacagacccugucacuauaagaguaaguucgacgucacaagucgugucgggcagcacuauaagagccggaggaaccggagguucuccauggagagguccugagccgacagugucuacuccgcaccaccccgcggguccugacccuccgggucucccucgcugucgucccuguccucuucggugucgguccguccuguaagcacguggggguagcacaguuccugccacucagugagaaccgugccccuuaggcgcaagguuacguggcaagggccggcgccuccgaccuagccagggccacagaagauaccuccaguuuugucgcaccuaccgcagagguccgcuagacagg

SEQ ID NO: 22 - RNA, 1802 nt, Artificial Sequence
  Chemically synthesized nucleotide
  misc_feature (901)..(902): 3'-3' bridge between nucleotides at positions 901 and 902 comprises PO4
ggacagaucgccuggagacgccauccacgcuguuuugaccuccauagaagacaccgggaccgauccagccuccgcggccgggaacggugcauuggaacgcggauuccccgugccaagagugacucaccguccuugacacgaugggggugcacgaauguccugccuggcuguggcuucuccugucccugcugucgcucccucugggccucccaguccugggcgccccaccacgccucaucugugacagccgaguccuggagagguaccucuuggaggccaaggaggccgagaauaucacgacgggcugugcugaacacugcagcuugaaugagaauaucacugucccagacaccaaaguuaauuucuaugccuggaagaggauggaggucgggcagcaggccguagaagucuggcagggccuggcccugcugucggaagcuguccugcggggccaggcccuguuggucaacucuucccagccgugggagccccugcagcugcauguggauaaagccgucaguggccuucgcagccucaccacucugcuucgggcucugggagcccagaaggaagccaucuccccuccagaugcggccucagcugcuccacuccgaacaaucacugcugacacuuuccgcaaacucuuccgagucuacuccaauuuccuccggggaaagcugaagcuguacacaggggaggccugcaggacaggggacagaugacggguggcaucccugugaccccuccccagugccucuccuggcccuggaaguugccacuccagugcccaccaaaaaaaaaaaaaaaaaaaaaaaaaaaaaaaaaaaaaaaaaaaaaaaaaaaaaaaaaaaaaaaaagccuuguccuaauaaaauuaaguugcaucaagcucgacucucggggcucucagcucgaacuacguugaauuaaaauaauccuguuccgaaaaaaaaaaaaaaaaaaaaaaaaaaaaaaaaaaaaaaaaaaaaaaaaaaaaaaaaaaaaaaaaaccacccgugaccucaccguugaaggucccgguccucuccgugaccccuccccagugucccuacggugggcaguagacaggggacaggacguccggaggggacacaugucgaagucgaaaggggccuccuuuaaccucaucugagccuucucaaacgccuuucacagucgucacuaacaagccucaccucgucgacuccggcguagaccuccccucuaccgaaggaagacccgagggucucgggcuucgucucaccacuccgacgcuuccggugacugccgaaauagguguacgucgacguccccgagggugccgacccuucucaacugguugucccggaccggggcguccugucgaaggcugucgucccgguccgggacggucugaagaugccggacgacgggcuggagguaggagaagguccguaucuuuaauugaaaccacagacccugucacuauaagaguaaguucgacgucacaagucgugucgggcagcacuauaagagccggaggaaccggagguucuccauggagagguccugagccgacagugucuacuccgcaccaccccgcggguccugacccuccgggucucccucgcugucgucccuguccucuucggugucgguccguccuguaagcacguggggguagcacaguuccugccacucagugagaaccgugccccuuaggcgcaagguuacguggcaagggccggcgccuccgaccuagccagggccacagaagauaccuccaguuuugucgcaccuaccgcagagguccgcuagacagg

SEQ ID NO: 23 - RNA, 1786 nt, Artificial Sequence
  Chemically synthesized nucleotide
  misc_feature (893)..(894): 3'-3' bridge between nucleotides at positions 893 and 894 comprises PO4
ggacagaucgccuggagacgccauccacgcuguuuugaccuccauagaagacaccgggaccgauccagccuccgcggccgggaacggugcauuggaacgcggauuccccgugccaagagugacucaccguccuugacacgaugggggugcacgaauguccugccuggcuguggcuucuccugucccugcugucgcucccucugggccucccaguccugggcgccccaccacgccucaucugugacagccgaguccuggagagguaccucuuggaggccaaggaggccgagaauaucacgacgggcugugcugaacacugcagcuugaaugagaauaucacugucccagacaccaaaguuaauuucuaugccuggaagaggauggaggucgggcagcaggccguagaagucuggcagggccuggcccugcugucggaagcuguccugcggggccaggcccuguuggucaacucuucccagccgugggagccccugcagcugcauguggauaaagccgucaguggccuucgcagccucaccacucugcuucgggcucugggagcccagaaggaagccaucuccccuccagaugcggccucagcugcuccacuccgaacaaucacugcugacacuuuccgcaaacucuuccgagucuacuccaauuuccuccggggaaagcugaagcuguacacaggggaggccugcaggacaggggacagaugacggguggcaaaaaaaaaaaaaaaucccugugaccccuccccaaaaaaaaaaaaaaaagugccucuccuggcccuggaaaaaaaaaaaaaaaguugccacuccagugcccaccaaaaaaaaaaaaaaagccuuguccuaauaaaauuaaguugcaucaagcucgacucucggggcucucagcucgaacuacguugaauuaaaauaauccuguuccgaaaaaaaaaaaaaaaccacccgugaccucaccguugaaaaaaaaaaaaaaaggucccgguccucuccgugaaaaaaaaaaaaaaaaccccuccccagugucccuaaaaaaaaaaaaaaacggugggcaguagacaggggacaggacguccggaggggacacaugucgaagucgaaaggggccuccuuuaaccucaucugagccuucucaaacgccuuucacagucgucacuaacaagccucaccucgucgacuccggcguagaccuccccucuaccgaaggaagacccgagggucucgggcuucgucucaccacuccgacgcuuccggugacugccgaaauagguguacgucgacguccccgagggugccgacccuucucaacugguugucccggaccggggcguccugucgaaggcugucgucccgguccgggacggucugaagaugccggacgacgggcuggagguaggagaagguccguaucuuuaauugaaaccacagacccugucacuauaagaguaaguucgacgucacaagucgugucgggcagcacuauaagagccggaggaaccggagguucuccauggagagguccugagccgacagugucuacuccgcaccaccccgcggguccugacccuccgggucucccucgcugucgucccuguccucuucggugucgguccguccuguaagcacguggggguagcacaguuccugccacucagugagaaccgugccccuuaggcgcaagguuacguggcaagggccggcgccuccgaccuagccagggccacagaagauaccuccaguuuugucgcaccuaccgcagagguccgcuagacagg

SEQ ID NO: 24 - RNA, 2640 nt, Artificial Sequence
  Chemically synthesized nucleotide
  misc_feature (1320)..(1321): 3'-3' bridge between nucleotides at positions 1320 and 1321 comprises PO4
ggacagaucgccuggagacgccauccacgcuguuuugaccuccauagaagacaccgggaccgauccagccuccgcggccgggaacggugcauuggaacgcggauuccccgugccaagagugacucaccguccuugacacgaugcuguucaaccuucggaucuugcugaacaacgcugcguuccggaauggucacaacuucaugguccggaacuucagaugcggccagccgcuccagaacaaggugcagcucaaggggagggaccuccucacccugaaaaacuucaccggagaagagaucaaguacaugcuguggcugucagccgaccucaaauuccggaucaagcagaagggcgaauaccuuccuuugcugcagggaaagucccuggggaugaucuucgagaagcgcagcacucgcacuagacugucaacugaaaccggcuucgcgcugcugggaggacaccccugcuuccugaccacccaagauauccaucugggugugaacgaaucccucaccgacacagcgcgggugcugucguccauggcagacgcgguccucgcccgcguguacaagcagucugaucuggacacucuggccaaggaagccuccauuccuaucauuaauggauuguccgaccucuaccaucccauccagauucuggccgauuaucugacucugcaagaacauuacagcucccugaaggggcuuacccuuucguggaucggcgacggcaacaacauucugcacagcauuaugaugagcgcugccaaguuuggaaugcaccuccaagcagcgaccccgaagggauacgagccagacgccuccgugacgaagcuggcugagcaguacgccaaggagaacggcacuaagcugcugcucaccaacgacccucucgaagccgcccacgguggcaacgugcugaucaccgauaccuggaucuccaugggacaggaggaggaaaagaagaagcgccugcaagcauuucagggguaccaggugacuaugaaaaccgccaaggucgccgccucggacuggaccuucuugcacugucugcccagaaagcccgaagagguggacgacgagguguucuacagcccgcggucgcuggucuuuccggaggccgaaaacaggaaguggacuaucauggccgugauggugucccugcugaccgauuacuccccgcagcugcagaaaccaaaguucugacggguggcaucccugugaccccuccccagugccucuccuggcccuggaaguugccacuccagugcccaccagccuuguccuaauaaaauuaaguugcaucaagcucgacucucggggcucucagcucgaacuacguugaauuaaaauaauccuguuccgaccacccgugaccucaccguugaaggucccgguccucuccgugaccccuccccagugucccuacggugggcagucuugaaaccaaagacgucgacgccccucauuagccagucgucccugugguagugccgguacuaucaggugaaggacaaaagccggaggccuuucuggucgcuggcgcccgacaucuuguggagcagcagguggagaagcccgaaagacccgucugucacguucuuccaggucaggcuccgccgcuggaaccgccaaaaguaucaguggaccauggggacuuuacgaacguccgcgaagaagaaaaggaggaggacaggguaccucuagguccauagccacuagucgugcaacgguggcacccgccgaagcucucccagcaaccacucgucgucgaaucacggcaagaggaaccgcaugacgagucggucgaagcagugccuccgcagaccgagcauagggaagccccagcgacgaaccuccacguaagguuugaaccgucgcgaguaguauuacgacacgucuuacaacaacggcagcggcuaggugcuuucccauucggggaagucccucgacauuacaagaacgucucagucuauuagccggucuuagaccuacccuaccaucuccagccuguuagguaauuacuauccuuaccuccgaaggaaccggucucacaggucuagucugacgaacaugugcgcccgcuccuggcgcagacgguaccugcugucgugggcgcgacacagccacucccuaagcaagugugggucuaccuauagaacccaccaguccuucguccccacaggagggucgucgcgcuucggccaaagucaacugucagaucacgcucacgacgcgaagagcuucuaguaggggucccugaaagggacgucguuuccuuccauaagcgggaagacgaacuaggccuuaaacuccagccgacugucggugucguacaugaacuagagaagaggccacuucaaaaagucccacuccuccagggaggggaacucgacguggaacaagaccucgccgaccggcguagacuucaaggccugguacuucaacacugguaaggccuugcgucgcaacaagucguucuaggcuuccaacuugucguagcacaguuccugccacucagugagaaccgugccccuuaggcgcaagguuacguggcaagggccggcgccuccgaccuagccagggccacagaagauaccuccaguuuugucgcaccuaccgcagagguccgcuagacagg

SEQ ID NO: 25 - RNA, 3228 nt, Artificial Sequence
  Chemically synthesized nucleotide
  misc_feature (1614)..(1615): 3'-3' bridge between nucleotides at positions 1614 and 1615 comprises PO4
ggacagaucgccuggagacgccauccacgcuguuuugaccuccauagaagacaccgggaccgauccagccuccgcggccgggaacggugcauuggaacgcggauuccccgugccaagagugacucaccguccuugacacgaugagcaccgccgugcuggagaaccccggccugggccgcaagcugagcgacuucggccaggagaccagcuacaucgaggacaacugcaaccagaacggcgccaucagccugaucuucagccugaaggaggaggugggcgcccuggccaaggugcugcgccuguucgaggagaacgacgugaaccugacccacaucgagagccgccccagccgccugaagaaggacgaguacgaguucuucacccaccuggacaagcgcagccugcccgcccugaccaacaucaucaagauccugcgccacgacaucggcgccaccgugcacgagcugagccgcgacaagaagaaggacaccgugcccugguucccccgcaccauccaggagcuggaccgcuucgccaaccagauccugagcuacggcgccgagcuggacgccgaccaccccggcuucaaggaccccguguaccgcgcccgccgcaagcaguucgccgacaucgccuacaacuaccgccacggccagcccaucccccgcguggaguacauggaggaggagaagaagaccuggggcaccguguucaagacccugaagagccuguacaagacccacgccugcuacgaguacaaccacaucuucccccugcuggagaaguacugcggcuuccacgaggacaacaucccccagcuggaggacgugagccaguuccugcagaccugcaccggcuuccgccugcgccccguggccggccugcugagcagccgcgacuuccugggcggccuggccuuccgcguguuccacugcacccaguacauccgccacggcagcaagcccauguacacccccgagcccgacaucugccacgagcugcugggccacgugccccuguucagcgaccgcagcuucgcccaguucagccaggagaucggccuggccagccugggcgcccccgacgaguacaucgagaagcuggccaccaucuacugguucaccguggaguucggccugugcaagcagggcgacagcaucaaggccuacggcgccggccugcugagcagcuucggcgagcugcaguacugccugagcgagaagcccaagcugcugccccuggagcuggagaagaccgccauccagaacuacaccgugaccgaguuccagccccuguacuacguggccgagagcuucaacgacgccaaggagaaggugcgcaacuucgccgccaccaucccccgccccuucagcgugcgcuacgaccccuacacccagcgcaucgaggugcuggacaacacccagcagcugaagauccuggccgacagcaucaacagcgagaucggcauccugugcagcgcccugcagaagaucaaguaacggguggcaucccugugaccccuccccagugccucuccuggcccuggaaguugccacuccagugcccaccagccuuguccuaauaaaauuaaguugcaucaagcucgacucucggggcucucagcucgaacuacguugaauuaaaauaauccuguuccgaccacccgugaccucaccguugaaggucccgguccucuccgugaccccuccccagugucccuacggugggcaaugaacuagaagacgucccgcgacguguccuacggcuagagcgacaacuacgacagccgguccuagaagucgacgacccacaacaggucguggagcuacgcgacccacauccccagcaucgcgugcgacuuccccgcccccuaccaccgccgcuucaacgcguggaagaggaaccgcagcaacuucgagagccggugcaucauguccccgaccuugagccagugccacaucaagaccuaccgccagaagaggucgagguccccgucgucgaacccgaagagcgaguccgucaugacgucgagcggcuucgacgagucguccggccgcggcauccggaacuacgacagcgggacgaacguguccggcuugaggugccacuuggucaucuaccaccggucgaagagcuacaugagcagcccccgcggguccgaccgguccggcuagaggaccgacuugacccgcuucgacgccagcgacuuguccccgugcaccgggucgucgagcaccgucuacagcccgagcccccacauguacccgaacgacggcaccgccuacaugacccacgucaccuugugcgccuuccgguccggcggguccuucagcgccgacgagucguccggccggugccccgcguccgccuucggccacguccagacguccuugaccgagugcaggaggucgacccccuacaacaggagcaccuucggcgucaugaagaggucgucccccuucuacaccaacaugagcaucguccgcacccagaacauguccgagaagucccagaacuugugccacgggguccagaagaagaggaggagguacaugaggugcgcccccuacccgaccggcaccgccaucaacauccgcuacagccgcuugacgaacgccgcccgcgccaugugccccaggaacuucggccccaccagccgcaggucgagccgcggcaucgaguccuagaccaaccgcuucgccaggucgaggaccuaccacgcccccuuggucccgugccacaggaagaagaacagcgccgagucgagcacgugccaccgcggcuacagcaccgcguccuagaacuacuacaaccagucccgcccguccgacgcgaacagguccacccacuucuugagcaugagcaggaagaaguccgccgaccccgccgagagcuacacccaguccaagugcagcaagaggagcuuguccgcgucguggaaccggucccgcggguggaggaggaaguccgacuucuaguccgacuaccgcggcaagaccaacgucaacaggagcuacaucgaccagaggaccggcuucagcgagucgaacgccggguccggccccaagaggucgugccgccacgaguagcacaguuccugccacucagugagaaccgugccccuuaggcgcaagguuacguggcaagggccggcgccuccgaccuagccagggccacagaagauaccuccaguuuugucgcaccuaccgcagagguccgcuagacagg

SEQ ID NO: 26 - RNA, 9396 nt, Artificial Sequence
  Chemically synthesized nucleotide
  misc_feature (4698)..(4699): 3'-3' bridge between nucleotides at positions 4698 and 14699 comprises PO4
ggacagaucgccuggagacgccauccacgcuguuuugaccuccauagaagacaccgggaccgauccagccuccgcggccgggaacggugcauuggaacgcggauuccccgugccaagagugacucaccguccuugacacgaugcaacgcucuccucuugaaaaggccucggugguguccaagcucuucuucucguggacuagacccauccugagaaagggguacagacagcgcuuggagcuguccgauaucuaucaaaucccuuccguggacuccgcggacaaccuguccgagaagcucgagagagaaugggacagagaacucgccucaaagaagaacccgaagcugauuaaugcgcuuaggcggugcuuuuucuggcgguucauguucuacggcaucuuccucuaccugggagaggucaccaaggccgugcagccccuguugcugggacggauuauugccuccuacgaccccgacaacaaggaagaaagaagcaucgcuaucuacuugggcaucggucugugccugcuuuucaucguccggacccucuuguugcauccugcuauuuucggccugcaucacauuggcaugcagaugagaauugccauguuuucccugaucuacaagaaaacucugaagcucucgagccgcgugcuugacaagauuuccaucggccagcucgugucccugcucuccaacaaucugaacaaguucgacgagggccucgcccuggcccacuucguguggaucgccccucugcaaguggcgcuucugaugggccugaucugggagcugcugcaagccucggcauucugugggcuuggauuccugaucgugcuggcacuguuccaggccggacuggggcggaugaugaugaaguacagggaccagagagccggaaagauuuccgaacggcuggugaucacuucggaaaugaucgaaaacauccagucagugaaggccuacugcugggaagaggccauggaaaagaugauugaaaaccuccggcaaaccgagcugaagcugacccgcaaggccgcuuacgugcgcuauuucaacucguccgcuuucuucuucuccggguucuucgugguguuucucuccgugcuccccuacgcccugauuaagggaaucauccucaggaagaucuucaccaccauuuccuucuguaucgugcuccgcauggccgugacccggcaguucccaugggccgugcagacuugguacgacucccugggagccauuaacaagauccaggacuuccuucaaaagcaggaguacaagacccucgaguacaaccugacuacuaccgaggucgugauggaaaacgucaccgccuuuugggaggagggauuuggcgaacuguucgagaaggccaagcagaacaacaacaaccgcaagaccucgaacggugacgacucccucuucuuuucaaacuucagccugcucgggacgcccgugcugaaggacauuaacuucaagaucgaaagaggacagcuccuggcgguggccggaucgaccggagccggaaagacuucccugcugauggugaucaugggagagcuugaaccuagcgagggaaagaucaagcacuccggccgcaucagcuucuguagccaguuuuccuggaucaugcccggaaccauuaaggaaaacaucaucuucggcguguccuacgaugaauaccgcuaccgguccgugaucaaagccugccagcuggaagaggauauuucaaaguucgcggagaaagauaacaucgugcugggcgaaggggguauuaccuugucggggggccagcgggcuagaaucucgcuggccagagccguguauaaggacgccgaccuguaucuccuggacucccccuucggauaccuggacguccugaccgaaaaggagaucuucgaaucgugcgugugcaagcugauggcuaacaagacucgcauccucgugaccuccaaaauggagcaccugaagaaggcagacaagauucugauucugcaugagggguccuccuacuuuuacggcaccuucucggaguugcagaacuugcagcccgacuucucaucgaagcugauggguugcgacagcuucgaccaguucuccgccgaaagaaggaacucgauccugacggaaaccuugcaccgcuucucuuuggaaggcgacgccccugugucauggaccgagacuaagaagcagagcuucaagcagaccggggaauucggcgaaaagaggaagaacagcaucuugaaccccauuaacuccauccgcaaguucucaaucgugcaaaagacgccacugcagaugaacggcauugaggaggacuccgacgaaccccuugagaggcgccugucccuggugccggacagcgagcagggagaagccauccugccucggauuuccgugaucuccacugguccgacgcuccaagcccggcggcggcaguccgugcugaaccugaugacccacagcgugaaccagggccaaaacauucaccgcaagacuaccgcauccacccggaaagugucccuggcaccucaagcgaaucuuaccgagcucgacaucuacucccggagacugucgcaggaaaccgggcucgaaauuuccgaagaaaucaacgaggaggaucugaaagagugcuucuucgacgauauggagucgauacccgccgugacgacuuggaacacuuaucugcgguacaucacugugcacaagucauugaucuucgugcugauuuggugccuggugauuuuccuggccgaggucgcggccucacugguggugcucuggcuguugggaaacacgccucugcaagacaagggaaacuccacgcacucgagaaacaacagcuaugccgugauuaucacuuccaccuccucuuauuacguguucuacaucuacgucggaguggcggauacccugcucgcgauggguuucuucagaggacugccgcugguccacaccuugaucaccgucagcaagauucuucaccacaagauguugcauagcgugcugcaggcccccauguccacccucaacacucugaaggccggaggcauucugaacagauucuccaaggacaucgcuauccuggacgaucuccugccgcuuaccaucuuugacuucauccagcugcugcugaucgugauuggagcaaucgcagugguggcggugcugcagccuuacauuuucguggccacugugccggucauuguggcguucaucaugcugcgggccuacuuccuccaaaccagccagcagcugaagcaacuggaauccgagggacgaucccccaucuucacucaccuugugacgucguugaagggacuguggacccuccgggcuuucggacggcagcccuacuucgaaacccucuuccacaaggcccugaaccuccacaccgccaauugguuccuguaccuguccacccugcggugguuccagaugcgcaucgagaugauuuucgucaucuucuucaucgcggucacauucaucagcauccugacuaccggagagggagagggacgggucggaauaauccugacccucgccaugaacauuaugagcacccugcagugggcagugaacagcucgaucgacguggacagccugaugcgaagcgucagccgcguguucaaguucaucgacaugccuacugagggaaaacccacuaaguccacuaagcccuacaaaaauggccagcugagcaaggucaugaucaucgaaaacucccacgugaagaaggacgauauuuggcccuccggaggucaaaugaccgugaaggaccugaccgcaaaguacaccgagggaggaaacgccauucucgaaaacaucagcuucuccauuucgccgggacagcgggucggccuucucgggcggaccgguuccgggaagucaacucugcugucggcuuuccuccggcugcugaauaccgagggggaaauccaaauugacggcgugucuugggauuccauuacucugcagcaguggcggaaggccuucggcgugaucccccagaagguguucaucuucucggguaccuuccggaagaaccuggauccuuacgagcaguggagcgaccaagaaaucuggaaggucgccgacgaggucggccugcgcuccgugauugaacaauuuccuggaaagcuggacuucgugcucgucgacgggggauguguccugucgcacggacauaagcagcucaugugccucgcacgguccgugcucuccaaggccaagauucugcugcuggacgaaccuucggcccaccuggauccggucaccuaccagaucaucaggaggacccugaagcaggccuuugccgauugcaccgugauucucugcgagcaccgcaucgaggccaugcuggagugccagcaguuccuggucaucgaggagaacaagguccgccaauacgacuccauucaaaagcuccucaacgagcggucgcuguucagacaagcuauuucaccguccgauagagugaagcucuucccgcaucggaacagcucaaagugcaaaucgaagccgcagaucgcagccuugaaggaagagacugaggaagaggugcaggacacccggcuuuaacggguggcaucccugugaccccuccccagugccucuccuggcccuggaaguugccacuccagugcccaccagccuuguccuaauaaaauuaaguugcaucaagcucgacucucggggcucucagcucgaacuacguugaauuaaaauaauccuguuccgaccacccgugaccucaccguugaaggucccgguccucuccgugaccccuccccagugucccuacggugggcaauuucggcccacaggacguggagaaggagucagagaaggaaguuccgacgcuagacgccgaagcuaaacgugaaacucgacaaggcuacgcccuucucgaagugagauagccugccacuuuaucgaacagacuugucgcuggcgagcaacuccucgaaaacuuaccucagcauaaccgccuggaacaagaggagcuacugguccuugacgaccgugaggucguaccggagcuacgccacgagcgucucuuagugccacguuagccguuuccggacgaagucccaggaggacuacuagaccauccacuggccuagguccacccggcuuccaagcaggucgucgucuuagaaccggaaccucucgugccuggcacgcuccguguacucgacgaauacaggcacgcuguccuguguagggggcagcugcucgugcuucaggucgaaagguccuuuaacaaguuagugccucgcguccggcuggagcagccgcuggaaggucuaaagaaccagcgaggugacgagcauuccuagguccaagaaggccuuccaugggcucuucuacuuguggaagacccccuagugcggcuuccggaaggcggugacgacgucucauuaccuuaggguucugugcggcaguuaaaccuaaagggggagccauaagucgucggccuccuuucggcugucgucucaacugaagggccuuggccaggcgggcucuuccggcugggcgacagggccgcuuuaccucuucgacuacaaaagcucuuaccgcaaaggagggagccacaugaaacgccaguccaggaagugccaguaaacuggaggccucccgguuuauagcaggaagaagugcacccucaaaagcuacuaguacuggaacgagucgaccgguaaaaacaucccgaaucaccugaaucacccaaaagggagucauccguacagcuacuugaacuugugcgccgacugcgaagcguaguccgacaggugcagcuagcucgacaagugacgggugacgucccacgaguauuacaaguaccgcucccaguccuaauaaggcugggcagggagagggagaggccaucaguccuacgacuacuuacacuggcgcuacuucuucuacugcuuuuaguagagcuacgcguagaccuugguggcgucccaccuguccauguccuugguuaaccgccacaccuccaagucccggaacaccuucucccaaagcuucaucccgacggcaggcuuucgggccucccaggugucagggaaguugcugcaguguuccacucacuucuacccccuagcagggagccuaaggucaacgaagucgacgaccgaccaaaccuccuucauccgggcgucguacuacuugcgguguuacuggccgugucaccggugcuuuuacauuccgacgucguggcgguggugacgcuaacgagguuagugcuagucgucgucgaccuacuucaguuucuaccauucgccguccucuagcagguccuaucgcuacaggaaccucuuagacaagucuuacggaggccggaagucucacaacucccaccuguacccccggacgucgugcgauacguuguagaacaccacuucuuagaacgacugccacuaguuccacaccuggucgccgucaggagacuucuuuggguagcgcucgucccauaggcggugaggcugcaucuacaucuugugcauuauucuccuccaccuucacuauuagugccguaucgacaacaaagagcucacgcaccucaaagggaacagaacgucuccgcacaaaggguugucggucucgugguggucacuccggcgcuggagccgguccuuuuagugguccgugguuuagucgugcuucuaguuacugaacacgugucacuacauggcgucuauucacaagguucagcagugccgcccauagcugagguauagcagcuucuucgugagaaagucuaggaggagcaacuaaagaagccuuuaaagcucgggccaaaggacgcugucagaggcccucaucuacagcucgagccauucuaagcgaacuccacggucccugugaaaggcccaccuacgccaucagaacgccacuuacaaaaccgggaccaagugcgacacccaguaguccaagucgugccugacggcggcggcccgaaccucgcagccuggucaccucuagugccuuuaggcuccguccuaccgaagagggacgagcgacaggccguggucccuguccgcggagaguuccccaagcagccucaggaggaguuacggcaaguagacgucaccgcagaaaacgugcuaacucuugaacgccuaccucaauuaccccaaguucuacgacaagaaggagaaaagcggcuuaaggggccagacgaacuucgagacgaagaaucagagccagguacuguguccccgcagcggaagguuucucuucgccacguuccaaaggcaguccuagcucaaggaagaaagccgccucuugaccagcuucgacagcguuggguagucgaagcuacucuucagcccgacguucaagacguugaggcucuuccacggcauuuucauccuccuggggaguacgucuuagucuuagaacagacggaagaaguccacgagguaaaaccuccagugcuccuacgcucagaacaaucgguagucgaacgugugcgugcuaagcuucuagaggaaaagccaguccugcagguccauaggcuucccccucagguccucuauguccagccgcaggaauaugugccgagaccggucgcucuaagaucgggcgaccggggggcuguuccauuaugggggaagcgggucgugcuacaauagaaagaggcgcuugaaacuuuauaggagaaggucgaccguccgaaacuagugccuggccaucgccauaaguagcauccugugcggcuucuacuacaaaaggaauuaccaaggcccguacuagguccuuuugaccgaugucuucgacuacgccggccucacgaacuagaaagggagcgauccaaguucgagaggguacuagugguagucgucccuucagaaaggccgaggccagcuaggccgguggcgguccucgacaggagaaagcuagaacuucaauuacaggaagucgugcccgcagggcucguccgacuucaaacuuuucuucucccucagcaguggcaagcuccagaacgccaacaacaacaagacgaaccggaagagcuugucaagcgguuuagggaggaggguuuuccgccacugcaaaagguagugcuggagccaucaucaguccaacaugagcucccagaacaugaggacgaaaacuuccuucaggaccuagaacaauuaccgagggucccucagcaugguucagacgugccggguacccuugacggcccagugccgguacgccucgugcuaugucuuccuuuaccaccacuucuagaaggacuccuacuaagggaauuagucccgcauccccucgugccucucuuuguggugcuucuugggccucuucuucuuucgccugcucaacuuuaucgcgugcauucgccggaacgcccagucgaagucgagccaaacggccuccaaaaguuaguagaaaagguaccggagaagggucgucauccggaagugacugaccuacaaaagcuaguaaaggcuucacuaguggucggcaagccuuuagaaaggccgagagaccagggacaugaaguaguaguaggcggggucaggccggaccuugucacggucgugcuaguccuuagguucgggugucuuacggcuccgaacgucgucgagggucuaguccggguagucuucgcggugaacgucuccccgcuaggugugcuucacccggucccgcuccgggagcagcuugaacaagucuaacaaccucucgucccugugcucgaccggcuaccuuuagaacaguucgugcgccgagcucucgaagucucaaaagaacaucuagucccuuuuguaccguuaagaguagacguacgguuacacuacguccggcuuuuaucguccuacguuguucucccaggccugcuacuuuucguccgugucuggcuacggguucaucuaucgcuacgaagaaagaaggaacaacagccccagcauccuccguuauuaggcagggucguuguccccgacgugccggaaccacuggagaggguccaucuccuucuacggcaucuuguacuuggcggucuuuuucguggcggauucgcguaauuagucgaagcccaagaagaaacuccgcucaagagacaggguaagagagagcucgaagagccuguccaacaggcgccucaggugccuucccuaaacuaucuauagccugucgagguucgcgacagacauggggaaagaguccuacccagaucaggugcucuucuucucgaaccugugguggcuccggaaaaguucuccucucgcaacguagcacaguuccugccacucagugagaaccgugccccuuaggcgcaagguuacguggcaagggccggcgccuccgaccuagccagggccacagaagauaccuccaguuuugucgcaccuaccgcagagguccgcuagacagg